European Patent Specification EP 3 009 509 B1, published August 30, 2023. Title: A heparosan-glucuronate-5-epimerase and a method for producing polysaccharide by using it. Applicant: Seikagaku Corporation. The sequence listing filed with the application follows.

SEQUENCE LISTING (42 sequences)

SEQ ID NO: 1 - DNA, 1806 bp, Achatina fulica
  CDS (1)..(1806)
atgcaccttacatgtgtaagaagagcctttcgtaaagttaactggctgcttcgttctgttgttctacttttgaccggaggatgtttgacaatattggtgaactggcaatggcccaatagtagaccatattattggctcagatcagatgcagagtttgctggacagtttgtatcaacggccgacagctctcagttgttcgaagatcaaacagtctcttgtccgccgtgtccaagtatagacgactttcctcagtcagcacaaactttggacctgcagataattaactgttcgataaatgaagcagagacaattgaatgtagacaagacaaaggagaagtctacatgccagtctccttcatcaacaactattttgaggtctttggagatgtgaaacgtgacggcaccagtaaactgtacaattttcagcatgcttacggcaagatccatccgccccagcctgtctatcacccaggaggggtattcctaaattttgagaagtacaatgtagcggctagagaaaagattctttgtgtgacagcttctgatggcgtgccattagccaaacagtgggatcccgctgggtactactacgccatttcagttgcacagtatggtctgagtcatcatgccaagggtattctagaaggaaacccaacgcccaggctgatggctggtggccaggtggaagagtcaaggtgggaaaatacaggccctgagatggaagttaatatcgcagagacaactgtagatggagaaatgatgagggtactgtcgttcagtgctccagaatcatatactgcccctggtcctgttcttcgtttgagcacgcaagagcagacaatctgttttgacttacaactgactggacctggtggggtcactgtacaaataaagaccaggaacggcagaacaggctacatacattttatccttgatgacagatacatggaggttaacggaagccacgttttatatggaataggcacgaagaatcttggaaaatgggtacatctaacaagagatatctttgtggactggatgaaaaccctgcataacgcacaattcagctcaccgacgcaattcaaagagatagtggatgtgacactgcatggaactgggtatcttgataacttaacattatctacatctgcgcacaacgaccatcttatccatgctgcgaactggctagttaataatcaagacagtgctggaggctggccaactagcattggaatgaaaaccggtgaaaacatcgaactgaaacctggctggtactccgctatgggtcaaggccaagcaatgtctacacttgtccgagcatataacctgactgcgcataaatattacctggataccgccgtacgagctttacatttatatgagttgggatctgatgttggtggtgttcgagctcgtttcctgggacaacttgattggtatgaggagtatccaaccacgccgaccagtaccttcgttctcaatggttttatttttgccatgcttggactttacgacgttatgaaaacagctgatggcgaaggacagcgagtagctgagaagttatggatgtcaggattgcactcactaaaagtgatgttgggtatgtatgattccggcacaggaacgctttatgatcttcgtcacataatcaaccacgaacagcctaatcgggccagatgggattatcatactacacatattgcgcttatccaggaaatggccatcattgacggtgaccctctgtttgacaccactgctaaaagatggatagattatttttacggcaaaagatctaagcacaattaa

SEQ ID NO: 2 - protein, 601 aa, Achatina fulica
MHLTCVRRAFRKVNWLLRSVVLLLTGGCLTILVNWQWPNSRPYYWLRSDAEFAGQFVSTADSSQLFEDQTVSCPPCPSIDDFPQSAQTLDLQIINCSINEAETIECRQDKGEVYMPVSFINNYFEVFGDVKRDGTSKLYNFQHAYGKIHPPQPVYHPGGVFLNFEKYNVAAREKILCVTASDGVPLAKQWDPAGYYYAISVAQYGLSHHAKGILEGNPTPRLMAGGQVEESRWENTGPEMEVNIAETTVDGEMMRVLSFSAPESYTAPGPVLRLSTQEQTICFDLQLTGPGGVTVQIKTRNGRTGYIHFILDDRYMEVNGSHVLYGIGTKNLGKWVHLTRDIFVDWMKTLHNAQFSSPTQFKEIVDVTLHGTGYLDNLTLSTSAHNDHLIHAANWLVNNQDSAGGWPTSIGMKTGENIELKPGWYSAMGQGQAMSTLVRAYNLTAHKYYLDTAVRALHLYELGSDVGGVRARFLGQLDWYEEYPTTPTSTFVLNGFIFAMLGLYDVMKTADGEGQRVAEKLWMSGLHSLKVMLGMYDSGTGTLYDLRHIINHEQPNRARWDYHTTHIALIQEMAIIDGDPLFDTTAKRWIDYFYGKRSKHN

SEQ ID NO: 3 - protein, 617 aa, Homo sapiens
MRCLAARVNYKTLIIICALFTLVTVLLWNKCSSDKAIQFPRRSSSGFRVDGFEKRAAASESNNYMNHVAKQQSEEAFPQEQQKAPPVVGGFNSNVGSKVLGLKYEEIDCLINDEHTIKGRREGNEVFLPFTWVEKYFDVYGKVVQYDGYDRFEFSHSYSKVYAQRAPYHPDGVFMSFEGYNVEVRDRVKCISGVEGVPLSTQWGPQGYFYPIQIAQYGLSHYSKNLTEKPPHIEVYETAEDRDKNKPNDWTVPKGCFMANVADKSRFTNVKQFIAPETSEGVSLQLGNTKDFIISFDLKFLTNGSVSVVLETTEKNQLFTIHYVSNAQLIAFKERDIYYGIGPRTSWSTVTRDLVTDLRKGVGLSNTKAVKPTKIMPKKVVRLIAKGKGFLDNITISTTAHMAAFFAASDWLVRNQDEKGGWPIMVTRKLGEGFKSLEPGWYSAMAQGQAISTLVRAYLLTKDHIFLNSALRATAPYKFLSEQHGVKAVFMNKHDWYEEYPTTPSSFVLNGFMYSLIGLYDLKETAGEKLGKEARSLYERGMESLKAMLPLYDTGSGTIYDLRHFMLGIAPNLARWDYHTTHINQLQLLSTIDESPVFKEFVKRWKSYLKGSRAKHN

SEQ ID NO: 4 - protein, 585 aa, Danio rerio
MRCLVARINHKTLIVICAVFALITILLWNKCSSDKDLPSPVRPLEFAAPTPEKEEENEGQAPEAPPGSREVAYEQIDCLINEDVLIKGRREGGEVYLPFSWVEKYFDVYGRLVQYDGMERFEFSHSYSRVYAQREPYHPDGVFMSFEGYNVEVRDRVKCISGVEGVPISTQWGPQGYFYPIQIAQYGLSHYSKNLTEKPPDIKIYGMLEEKEGGSSQWDVPKGCTLSKIQDQGRSGFVHHFVTAENSEGVSLVLDNAKDFVLTFDVKFISNGSVSVVLETTEKGPYFIIHYITSPLLLSFKDREVIYGIGPRATWSTVSRDLVTDLRKGVGLSNTKVVKATKIMPRRVVQLVLKGSGFISNITVSSTAHMAAFFAASDWLLHNQDEHGGWPIKVTRKLGEGFKSLEPGWYSAMAQGQAMSTLVRAYLVTHNPSYLGAAIRATSPFKRTPEQHGVKATFMNKFDWYEEYPTTPSSFVLNGFIYSLIGLYDVAETAGNKLGREAGILFSQGLESLKAMLPLFDTGSGTVYDLRHFTLGVAPNLARWDYHTTHINQLQLLASIDGAPIFRDYVKRWKTYLKGGRAKHN

SEQ ID NO: 5 - protein, 616 aa, Caenorhabditis elegans
MKCLRWRSNRHRIYLLVACGALFLLNRHLTQEESRIDEEDEELTQVDVNEDDKKIECEPPGSIESKCIADNGKSMKCWKDEEDVYFPVSYLKKRFDMTGKLGKDGSTFELYTSYAKMRSPDSTYDPLGPFGHFSTYSVETRDRVRCVSAKTDVPMSTQWDPIPYYYPIQISQYGLQHYSRMKLDSISNKSEASPKDDVILGVNSKEWKGAAGMHETTERLFFNDEQMGKVVNISAGAALANAGAYVYLDKSPDLHVISFDWKPYEANSSFTVLAKMKQDDLLVLINYVYSEGNGKCVWQEEERISDDYIVQKPKKDGQVSYSYSYIGNSPIGEWSTVTRDLLVDVARALSSGDNRKKDDNVVLHAGDLRLVSLGFRGELTVKQKITQRREQHSHAFYAAADWLVKNQNDRGGWSVPVERSIAERKLVLPPGWHSAMAQGHGISVLTRAFKHFNDEKYLKSAAKALKLFKINSSDGGVRGEFFGNIWYEEYPTTPGSFVLNGFLYSLIGLYDLSQLELMIDENDETMRAKIQEAQELYSAGVRSLKQLLPLYDTGSGTIYDLRHVALGTAPNLARWDYHAVHVYLLKWIAGIEKDEVLSKTADRWIGYAYGKRAKHN

SEQ ID NO: 6 - DNA, 50 bp, Artificial Sequence
  designed oligo-dT primer bearinig a XhoI site for reverse transcription
gagagagagagagagagagaactagtctcgagtttttttttttttttttt

SEQ ID NO: 7 - DNA, 14 bp, Artificial Sequence
  designed sense oligo-nucleotide of EcoRI adaptor
aattcggcacgagg

SEQ ID NO: 8 - DNA, 10 bp, Artificial Sequence
  designed anti-sense oligo-nucleotide of EcoRI adaptor
cctcgtgccg

SEQ ID NO: 9 - DNA, 20 bp, Artificial Sequence
  designed sense primer for PCR cloning of heparosan-glucuronate-5-epimerase
tggtatgaggaatatccaac

SEQ ID NO: 10 - DNA, 20 bp, Artificial Sequence
  designed sense primer for PCR cloning of heparosan-glucuronate-5-epimerase
tcttttgtgctcaatggatt

SEQ ID NO: 11 - DNA, 26 bp, Artificial Sequence
  designed sense primer for PCR cloning of heparosan-glucuronate-5-epimerase
tattcacttattggactttatgatct

SEQ ID NO: 12 - DNA, 17 bp, Artificial Sequence
  designed anti-sense primer for PCR cloning of heparosan-glucuronate-5-epimerase
ttaattatgttttgccc

SEQ ID NO: 13 - DNA, 24 bp, Artificial Sequence
  designed anti-sense primer for PCR cloning of heparosan-glucuronate-5-epimerase
atgataatcccatcttgcaagatt

SEQ ID NO: 14 - DNA, 20 bp, Artificial Sequence
  designed sense primer for insert check PCR named as T3 primer
aattaaccctcactaaaggg

SEQ ID NO: 15 - DNA, 20 bp, Artificial Sequence
  designed anti-sense primer for insert check PCR named as T7 primer
taatacgactcactataggg

SEQ ID NO: 16 - DNA, 255 bp, Achatina fulica
tggtatgaggaatatccaaccacgccgaccagtaccttcgttctcaatggttttatttttgccatgcttggactttacgacgttatgaaaacagctgatggcgaaggacagcgagtagctgagaagttatggatgtcaggattgcactcactaaaagtgatgttgggtatgtatgattccggcacaggaacgctttatgatcttcgtcacataatcaaccacgaacagcctaatcttgcaagatgggattatcat

SEQ ID NO: 17 - DNA, 20 bp, Artificial Sequence
  designed sense primer for inverse PCR
tggatgtcaggattgcactc

SEQ ID NO: 18 - DNA, 20 bp, Artificial Sequence
  designed anti-sense primer for inverse PCR
cttcgccatcagctgttttc

SEQ ID NO: 19 - DNA, 20 bp, Artificial Sequence
  designed sense primer for nested PCR
ggtatgtatgattccggcac

SEQ ID NO: 20 - DNA, 20 bp, Artificial Sequence
  designed anti-sense primer for nested PCR
tcgtaaagtccaagcatggc

SEQ ID NO: 21 - DNA, 20 bp, Artificial Sequence
  designed sense primer for PCR cloning of heparosan-glucuronate-5-epimerase
tgatgagggtactgtcgttc

SEQ ID NO: 22 - DNA, 23 bp, Artificial Sequence
  designed anti-sense primer for PCR cloning of heparosan-glucuronate-5-epimerase
ttaattgtgcttagatcttttgc

SEQ ID NO: 23 - DNA, 1049 bp, Achatina fulica
tgatgagggtactgtcgttcagtgctccagaatcatatactgcccctggtcctgttcttcgtttgagcacgcaagagcagacaatctgttttgacttacaactgactggacctggtggggtcactgtacaaataaagaccaggaacggcagaacaggctacatacattttatccttgatgacagatacatggaggttaacggaagccacgttttatatggaataggcacgaagaatcttggaaaatgggtacatctaacaagagatatctttgtggactggatgaaaaccctgcataacgcacaattcagctcaccgacgcaattcaaagagatagtggatgtgacactgcatggaactgggtatcttgataacttaacattatctacatctgcgcacaacgaccatcttatccatgctgcgaactggctagttaataatcaagacagtgctggaggctggccaactagcattggaatgaaaaccggtgaaaacatcgaactgaaacctggctggtactccgctatgggtcaaggccaagcaatgtctacacttgtccgagcatataacctgactgcgcataaatattacctggataccgccgtacgagctttacatttatatgagttgggatctgatgttggtggtgttcgagctcgtttcctgggacaacttgattggtatgaggagtatccaaccacgccgaccagtaccttcgttctcaatggttttatttttgccatgcttggactttacgacgttatgaaaacagctgatggcgaaggacagcgagtagctgagaagttatggatgtcaggattgcactcactaaaagtgatgttgggtatgtatgattccggcacaggaacgctttatgatcttcgtcacataatcaaccacgaacagcctaatcgggccagatgggattatcatactacacatattgcgcttatccaggaaatggccatcattgacggtgaccctctgtttgacaccactgctaaaagatggatagattatttttacggcaaaagatctaagcacaattaa

SEQ ID NO: 24 - DNA, 27 bp, Artificial Sequence
  designed sense primer for 5' RACE of heparosan-glucuronate-5-epimerase
ccatcctaatacgactcactatagggc

SEQ ID NO: 25 - DNA, 25 bp, Artificial Sequence
  designed anti-sense primer for 5' RACE of heparosan-glucuronate-5-epimerase
cattgcttggccttgacccatagcg

SEQ ID NO: 26 - DNA, 23 bp, Artificial Sequence
  designed sense primer for nested PCR
actcactatagggctcgagcggc

SEQ ID NO: 27 - DNA, 26 bp, Artificial Sequence
  designed anti-sense primer for nested PCR
tctctttgaattgcgtcggtgagctg

SEQ ID NO: 28 - DNA, 1200 bp, Achatina fulica
actcactatagggctcgagcggccgcccgggcaggtatttgaatattctcacttattccaggattttcagtttttatcgcatgtttgttacaacactcactggagaggatatgcaccttacatgtgtaagaagagcctttcgtaaagttaactggctgcttcgttctgttgttctacttttgaccggaggatgtttgacaatattggtgaactggcaatggcccaatagtagaccatattattggctcagatcagatgcagagtttgctggacagtttgtatcaacggccgacagctctcagttgttcgaagatcaaacagtctcttgtccgccgtgtccaagtatagacgactttcctcagtcagcacaaactttggacctgcagataattaactgttcgataaatgaagcagagacaattgaatgtagacaagacaaaggagaagtctacatgccagtctccttcatcaacaactattttgaggtctttggagatgtgaaacgtgacggcaccagtaaactgtacaattttcagcatgcttacggcaagatccatccgccccagcctgtctatcacccaggaggggtattcctaaattttgagaagtacaatgtagcggctagagaaaagattctttgtgtgacagcttctgatggcgtgccattagccaaacagtgggatcccgctgggtactactacgccatttcagttgcacagtatggtctgagtcatcatgccaagggtattctagaaggaaacccaacgcccaggctgatggctggtggccaggtggaagagtcaaggtgggaaaatacaggccctgagatggaagttaatatcgcagagacaactgtagatggagaaatgatgagggtactgtcgttcagtgctccagaatcatatactgcccctggtcctgttcttcgtttgagcacgcaagagcagacaatctgttttgacttacaactgactggacctggtggggtcactgtacaaataaagaccaggaacggcagaacaggctacatacattttatccttgatgacagatacatggaggttaacggaagccacgttttatatggaataggcacgaagaatcttggaaaatgggtacatctaacaagagatatctttgtggactggatgaaaaccctgcataacgcacaattcagctcaccgacgcaattcaaagaga

SEQ ID NO: 29 - DNA, 30 bp, Artificial Sequence
  designed sense primer for preparation of an expression vector encoding heparosan-glucuronate-5-epimerase
acagaattctaactggcaatggcccaatag

SEQ ID NO: 30 - DNA, 34 bp, Artificial Sequence
  designed anti-sense primer for preparation of an expression vector encoding heparosan-glucuronate-5-epimerase
tgtgcggccgcttaattgtgcttagatcttttgc

SEQ ID NO: 31 - protein, 22 aa, Artificial Sequence
  secretion signal peptide of the kappa-chain of mouse immunoglobulin
MHFQVQIFSFLLISASVIMSRG

SEQ ID NO: 32 - protein, 8 aa, Artificial Sequence
  FLAG peptide
DYKDDDDK

SEQ ID NO: 33 - DNA, 90 bp, Artificial Sequence
  recombinant DNA sequence encoding secretion signal peptide of the kappa-chain of mouse immunoglobulin and FLAG peptide
  CDS (1)..(90)
atgcattttcaagtgcagattttcagcttcctgctaatcagtgcctcagtcataatgtcacgtggagattacaaggacgacgatgacaag

SEQ ID NO: 34 - protein, 30 aa, Artificial Sequence
  fusion peptide comprising of secretion signal peptide of the kappa-chain of mouse immunoglobulin and FLAG peptide
MHFQVQIFSFLLISASVIMSRGDYKDDDDK

SEQ ID NO: 35 - DNA, 36 bp, Artificial Sequence
  designed sense primer for preparation of an expression vector named as pFBIF1
acaggatccaccatgcattttcaagtgcagattttc

SEQ ID NO: 36 - DNA, 50 bp, Artificial Sequence
  designed anti-sense primer for preparation of an expression vector named as pFBIF1
acagaattcttgtcatcgtcgtccttgtaatctccacgtgacattatgac

SEQ ID NO: 37 - DNA, 29 bp, Artificial Sequence
  designed sense primer for preparation of an expression vector encoding heparosan-glucuronate-5-epimerase
acagtcgacaactggcaatggcccaatag

SEQ ID NO: 38 - DNA, 26 bp, Artificial Sequence
  designed anti-sense primer for preparation of an expression vector encoding heparosan-glucuronate-5-epimerase
acaggtaccttaattgtgcttagatc

SEQ ID NO: 39 - DNA, 23 bp, Artificial Sequence
  designed sense primer for preparation of an expression vector named as pFBIF2
acagaattccaccatgcattttc

SEQ ID NO: 40 - DNA, 28 bp, Artificial Sequence
  designed anti-sense primer for preparation of an expression vector named as pFBIF2
acagtcgaccttgtcatcgtcgtccttg

SEQ ID NO: 41 - DNA, 17 bp, Artificial Sequence
  designed sense primer for insert check PCR named as M13 Forward (-40)
gttttcccagtcacgac

SEQ ID NO: 42 - DNA, 17 bp, Artificial Sequence
  designed anti-sense primer for insert check PCR named as M13 Reverse
caggaaacagctatgac